European Patent Specification EP 3 897 156 B1, published July 9, 2025. Title: Microbacterium esteraromaticum strain, composition comprising the same, and uses thereof. Applicant: Futureco Bioscience SA. The sequence listing filed with the application follows.

SEQUENCE LISTING (7 sequences)

SEQ ID NO: 1 - DNA, 18 bp, Artificial Sequence
  oligonuclotide for 16S rRNA sequencing
agtttgatcctggctcag

SEQ ID NO: 2 - DNA, 21 bp, Artificial Sequence
  oligonucleotide for 16S rRNA sequencing
acggttaccttgttacgactt

SEQ ID NO: 3 - DNA, 970 bp, Artificial Sequence
  amplicon
tgcaagtcgaacgatgaagcccagcttgctgggtggattagtggcgaacgggtgagtaacacgtgagcaacctgcccctgactctgggataagcgctggaaacggcgtctaatactggatatgtcccgtcaccgcatggtgtgcgggtggaaagatttttcggttggggatgggctcgcggcctatcagcttgttggtgaggtaatggctcaccaaggcgtcgacgggtagccggcctgagagggtgaccggccacactgggactgagacacggcccagactcctacgggaggcagcagtggggaatattgcacaatgggcggaagcctgatgcagcaacgccgcgtgagggatgacggccttcgggttgtaaacctcttttagcagggaagaagcgaaagtgacggtacctgcagaaaaagcaccggctaactacgtgccagcagccgcggtaatacgtagggtgcaagcgttatccggaattattgggcgtaaagagctcgtaggcggtctgtcgcgtctgctgtgaaatcccgaggctcaacctcgggcttgcagtgggtacgggcagactagagtgcggtaggggagattggaattcctggtgtagcggtggaatgcgcagatatcaggaggaacaccgatggcgaaggcagatctctgggccgtaactgacgctgaggagcgaaagggtggggagcaaacaggcttagataccctggtagtccaccccgtaaacgttgggaactagttgtggggtcctttccacggattccgtgacgcagctaacgcattaagttccccgcctggggagtacggccgcaaggctaaaactcaaaggaattgacggggacccgcacaagcggcggagcatgcggattaattcgatgcaacgcgaagaaccttaccaaggcttgacatacacgagaacgggccagaaatggtcaactctttggacactcgtgaacag

SEQ ID NO: 4 - DNA, 20 bp, Artificial Sequence
  primer
cctcgttctatgttgccagc

SEQ ID NO: 5 - DNA, 20 bp, Artificial Sequence
  primer reverse
tgcagacctcaatccgaact

SEQ ID NO: 6 - DNA, 20 bp, Artificial Sequence
  Primer forward
ctgggataagcgctggaaac

SEQ ID NO: 7 - DNA, 20 bp, Artificial Sequence
  primer reverse
caatattccccactgctgcc